European Patent Specification EP 4 211 263 B1, published December 11, 2024. Title: CYTOSINE MODIFICATION ANALYSIS. Applicant: THE CHANCELLOR, MASTERS AND SCHOLARS OF THE UNIVERSITY OF OXFORD. The sequence listing filed with the application follows.

SEQUENCE LISTING (6 sequences)

SEQ ID NO: 1 - DNA, 74 bp, Artificial sequence
  Synthetic
agagagcaagccggctatagatgctacgtacagtagcagctgatcaagactgctaaggccacaaccagttggcg

SEQ ID NO: 2 - DNA, 90 bp, Artificial sequence
  Synthetic
actctcactctcacctccatcttacttgtctaccgaatcctcacgtactcacgattcgaccatccacattcgccaacuggutguggcctt

SEQ ID NO: 3 - DNA, 144 bp, Artificial sequence
  Synthetic
agagagcaagccggctatagatgctacgtacagtagcagctgatcaagactgctaaggccacaaccagttggcgaatgtggatggtcgaatcgtgagtacgtgaggattcggtagacaagtaagatggaggtgagagtgagagt

SEQ ID NO: 4 - DNA, 22 bp, Artificial sequence
  Forward Primer
actggaacaacactcaacccta

SEQ ID NO: 5 - DNA, 22 bp, Artificial sequence
  Reverse Primer
agagcagattgtactgagagtg

SEQ ID NO: 6 - DNA, 2026 bp, Artificial sequence
  Synthetic
actggaacaacactcaaccctatctcggtctattcttttgatttataagggattttgccgatttcggcctattggttaaaaaatgagctgatttaacaaaaatttaacgcgaattttaacaaaatattaacgtttacaatttcaggtggcacttttcggggaaatgtgcgcggaacccctatttgtttatttttctaaatacattcaaatatgtatccgctcatgaattaattcttagaaaaactcatcgagcatcaaatgaaactgcaatttattcatatcaggattatcaataccatatttttgaaaaagccgtttctgtaatgaaggagaaaactcaccgaggcagttccataggatggcaagatcctggtatcggtctgcgattccgactcgtccaacatcaatacaacctattaatttcccctcgtcaaaaataaggttatcaagtgagaaatcaccatgagtgacgactgaatccggtgagaatggcaaaagtttatgcatttctttccagacttgttcaacaggccagccattacgctcgtcatcaaaatcactcgcatcaaccaaaccgttattcattcgtgattgcgcctgagcgagacgaaatacgcgatcgctgttaaaaggacaattacaaacaggaatcgaatgcaaccggcgcaggaacactgccagcgcatcaacaatattttcacctgaatcaggatattcttctaatacctggaatgctgttttcccggggatcgcagtggtgagtaaccatgcatcatcaggagtacggataaaatgcttgatggtcggaagaggcataaattccgtcagccagtttagtctgaccatctcatctgtaacatcattggcaacgctacctttgccatgtttcagaaacaactctggcgcatcgggcttcccatacaatcgatagattgtcgcacctgattgcccgacattatcgcgagcccatttatacccatataaatcagcatccatgttggaatttaatcgcggcctagagcaagacgtttcccgttgaatatggctcataacaccccttgtattactgtttatgtaagcagacagttttattgttcatgaccaaaatcccttaacgtgagttttcgttccactgagcgtcagaccccgtagaaaagatcaaaggatcttcttgagatcctttttttctgcgcgtaatctgctgcttgcaaacaaaaaaaccaccgctaccagcggtggtttgtttgccggatcaagagctaccaactctttttccgaaggtaactggcttcagcagagcgcagataccaaatactgtccttctagtgtagccgtagttaggccaccacttcaagaactctgtagcaccgcctacatacctcgctctgctaatcctgttaccagtggctgctgccagtggcgataagtcgtgtcttaccgggttggactcaagacgatagttaccggataaggcgcagcggtcgggctgaacggggggttcgtgcacacagcccagcttggagcgaacgacctacaccgaactgagatacctacagcgtgagctatgagaaagcgccacgcttcccgaagggagaaaggcggacaggtatccggtaagcggcagggtcggaacaggagagcgcacgagggagcttccagggggaaacgcctggtatctttatagtcctgtcgggtttcgccacctctgacttgagcgtcgatttttgtgatgctcgtcaggggggcggagcctatggaaaaacgccagcaacgcggcctttttacggttcctggccttttgctggccttttgctcacatgttctttcctgcgttatcccctgattctgtggataaccgtattaccgcctttgagtgagctgataccgctcgccgcagccgaacgaccgagcgcagcgagtcagtgagcgaggaagcggaagagcgcctgatgcggtattttctccttacgcatctgtgcggtatttcacaccgcatatatggtgcactctcagtacaatctgctct